European Patent Application EP 4 613 765 A1, published September 10, 2025. Title: PROTEIN COMPOSITIONS AND CONSUMABLE PRODUCTS THEREOF. Applicant: CLARA FOODS CO. The sequence listing filed with the application follows.

SEQUENCE LISTING (53 sequences)

SEQ ID NO: 1 - protein, 186 aa, Gallus gallus
AEVDCSRFPNATDKEGKDVLVCNKDLRPICGTDGVTYTNDCLLCAYSIEFGTNISKEHDGECKETVPMNCSSYANTTSEDGKVMVLCNRAFNPVCGTDGVTYDNECLLCAHKVEQGASVDKRHDGGCRKELAAVSVDCSEYPKPDCTAEDRPLCGSDNKTYGNKCNFCNAVVESNGTLTLSHFGKC

SEQ ID NO: 2 - protein, 186 aa, Gallus gallus
AEVDCSRFPNATDMEGKDVLVCNKDLRPICGTDGVTYTNDCLLCAYSVEFGTNISKEHDGECKETVPMNCSSYANTTSEDGKVMVLCNRAFNPVCGTDGVTYDNECLLCAHKVEQGASVDKRHDGGCRKELAAVSVDCSEYPKPDCTAEDRPLCGSDNKTYGNKCNFCNAVVESNGTLTLSHFGKC

SEQ ID NO: 3 - protein, 186 aa, Gallus gallus
AEVDCSRFPNATDMEGKDVLVCNKDLRPICGTDGVTYTNDCLLCAYSVEFGTNISKEHDGECKETVPMNCSSYANTTSEDGKVMVLCNRAFNPVCGTDGVTYDNECLLCAHKVEQGASVDKRHDGGCRKELAAVSVDCSEYPKPDCTAEDRPLCGSDNKTYMNKCNACNAVVESNGTLTLSHFGKC

SEQ ID NO: 4 - protein, 210 aa, Gallus gallus
MAMAGVFVLFSFVLCGFLPDAAFGAEVDCSRFPNATDKEGKDVLVCNKDLRPICGTDGVTYTNDCLLCAYSIEFGTNISKEHDGECKETVPMNCSSYANTTSEDGKVMVLCNRAFNPVCGTDGVTYDNECLLCAHKVEQGASVDKRHDGGCRKELAAVSVDCSEYPKPDCTAEDRPLCGSDNKTYGNKCNFCNAVVESNGTLTLSHFGKC

SEQ ID NO: 5 - protein, 210 aa, Gallus gallus
MAMAGVFVLFSFVLCGFLPDAVFGAEVDCSRFPNATDMEGKDVLVCNKDLRPICGTDGVTYTNDCLLCAYSVEFGTNISKEHDGECKETVPMNCSSYANTTSEDGKVMVLCNRAFNPVCGTDGVTYDNECLLCAHKVEQGASVDKRHDGGCRKELAAVSVDCSEYPKPDCTAEDRPLCGSDNKTYGNKCNFCNAVVESNGTLTLSHFGKC

SEQ ID NO: 6 - protein, 208 aa, Gallus gallus
MAMAGVFVLFSFVLCGFLPDAAFGAEVDCSRFPNATDKEGKDVLVCNKDLRPICGTDGVTYTNDCLLCAYSIEFGTNISKEHDGECKETVPMNCSSYANTTSEDGKVMVLCNRAFNPVCGTDGVTYDNECLLCAHKVEQGASVDKRHDGGCRKELAAVDCSEYPKPDCTAEDRPLCGSDNKTYGNKCNFCNAVVESNGTLTLSHFGKC

SEQ ID NO: 7 - protein, 186 aa, Gallus gallus
AEVDCSRFPNATDKEGKDVLVCNKDLRPICGTDGVTYNNECLLCAYSIEFGTNISKEHDGECKETVPMNCSSYANTTSEDGKVMVLCNRAFNPVCGTDGVTYDNECLLCAHKVEQGASVDKRHDGECRKELAAVSVDCSEYPKPDCTAEDRPLCGSDNKTYGNKCNFCNAVVESNGTLTLSHFGKC

SEQ ID NO: 8 - protein, 208 aa, Numida meleagris
MAMAGVFVLFSFALCGFLPDAAFGVEVDCSRFPNATNEEGKDVLVCTEDLRPICGTDGVTYSNDCLLCAYNIEYGTNISKEHDGECREAVPVDCSRYPNMTSEEGKVLILCNKAFNPVCGTDGVTYDNECLLCAHNVEQGTSVGKKHDGECRKELAAVDCSEYPKPACTMEYRPLCGSDNKTYDNKCNFCNAVVESNGTLTLSHFGKC

SEQ ID NO: 9 - protein, 239 aa, Meleagris gallopavo
MQTITWRQPQGDHLRSRAPAATCRAGQYLTMAMAGIFVLFSFALCGFLPDAAFGVEVDCSRFPNTTNEEGKDVLVCTEDLRPICGTDGVTHSECLLCAYNIEYGTNISKEHDGECREAVPMDCSRYPNTTNEEGKVMILCNKALNPVCGTDGVTYDNECVLCAHNLEQGTSVGKKHDGGCRKELAAVSVDCSEYPKPACTLEYRPLCGSDNKTYGNKCNFCNAVVESNGTLTLSHFGKC

SEQ ID NO: 10 - protein, 185 aa, Meleagris gallopavo
VEVDCSRFPNTTNEEGKDVLVCTEDLRPICGTDGVTHSECLLCAYNIEYGTNISKEHDGECREAVPMDCSRYPNTTSEEGKVMILCNKALNPVCGTDGVTYDNECVLCAHNLEQGTSVGKKHDGECRKELAAVSVDCSEYPKPACTLEYRPLCGSDNKTYGNKCNFCNAVVESNGTLTLSHFGKC

SEQ ID NO: 11 - protein, 237 aa, Meleagris gallopavo
MQTITWRQPQGDHLRSRAPAATCRAGQYLTMAMAGIFVLFSFALCGFLPDAAFGVEVDCSRFPNTTNEEGKDVLVCTEDLRPICGTDGVTHSECLLCAYNIEYGTNISKEHDGECREAVPMDCSRYPNTTNEEGKVMILCNKALNPVCGTDGVTYDNECVLCAHNLEQGTSVGKKHDGGCRKELAAVDCSEYPKPACTLEYRPLCGSDNKTYGNKCNFCNAVVESNGTLTLSHFGKC

SEQ ID NO: 12 - protein, 128 aa, Bambusicola thoracicus
EYGTNISIKHNGECKETVPMDCSRYANMTNEEGKVMMPCDRTYNPVCGTDGVTYDNECQLCAHNVEQGTSVDKKHDGVCGKELAAVSVDCSEYPKPECTAEERPICGSDNKTYGNKCNFCNAVVYVQP

SEQ ID NO: 13 - protein, 195 aa, Callipepla squamata
VDCSRFPNTTNEEGKDVLACTKELHPICGTDGVTYSNECLLCYYNIEYGTNISKEHDGECTEAVPVDCSRYPNTTSEEGKVLIPCNRDFNPVCGSDGVTYENECLLCAHNVEQGTSVGKKHDGGCRKEFAAVSVDCSEYPKPDCTLEYRPLCGSDNKTYASKCNFCNAVVIWEQEKNTRHHASHSVFFISARLVC

SEQ ID NO: 14 - protein, 339 aa, Colinus virginianus
MLPLGLREYGTNTSKEHDGECTEAVPVDCSRYPNTTSEEGKVRILCKKDINPVCGTDGVTYDNECLLCSHSVGQGASIDKKHDGGCRKEFAAVSVDCSEYPKPACMSEYRPLCGSDNKTYVNKCNFCNAVVYVQPWLHSRCRLPPTGTSFLGSEGRETSLLTSRATDLQVAGCTAISAMEATRAAALLGLVLLSSFCELSHLCFSQASCDVYRLSGSRNLACPRIFQPVCGTDNVTYPNECSLCRQMLRSRAVYKKHDGRCVKVDCTGYMRATGGLGTACSQQYSPLYATNGVIYSNKCTFCSAVANGEDIDLLAVKYPEEESWISVSPTPWRMLSAGA

SEQ ID NO: 15 - protein, 238 aa, Anser cygnoides
  source 1..238: note = Anser cygnoides domesticus
MSWWGIKPALERPSQEQSTSGQPVDSGSTSTTTMAGIFVLLSLVLCCFPDAAFGVEVDCSRFPNTTNEEGKEVLLCTKDLSPICGTDGVTYSNECLLCAYNIEYGTNISKDHDGECKEAVPVDCSTYPNMTNEEGKVMLVCNKMFSPVCGTDGVTYDNECMLCAHNVEQGTSVGKKYDGKCKKEVATVDCSDYPKPACTVEYMPLCGSDNKTYDNKCNFCNAVVDSNGTLTLSHFGKC

SEQ ID NO: 16 - protein, 284 aa, Anser cygnoides
  source 1..284: note = Anser cygnoides domesticus
MSSQNQLHRRRRPLPGGQDLNKYYWPHCTSDRFSWLLHVTAEQFRHCVCIYLQPALERPSQEQSTSGQPVDSGSTSTTTMAGIFVLLSLVLCCFPDAAFGVEVDCSRFPNTTNEEGKEVLLCTKDLSPICGTDGVTYSNECLLCAYNIEYGTNISKDHDGECKEAVPVDCSTYPNMTNEEGKVMLVCNKMFSPVCGTDGVTYDNECMLCAHNVEQGTSVGKKYDGKCKKEVATVDCSDYPKPACTVEYMPLCGSDNKTYDNKCNFCNAVVDSNGTLTLSHFGKC

SEQ ID NO: 17 - protein, 186 aa, Coturnix japonica
VEVDCSRFPNTTNEEGKDEVVCPDELRLICGTDGVTYNHECMLCFYNKEYGTNISKEQDGECGETVPMDCSRYPNTTSEDGKVTILCTKDFSFVCGTDGVTYDNECMLCAHNVVQGTSVGKKHDGECRKELAAVSVDCSEYPKPACPKDYRPVCGSDNKTYSNKCNFCNAVVESNGTLTLNHFGKC

SEQ ID NO: 18 - protein, 210 aa, Coturnix japonica
MAMAGVFLLFSFALCGFLPDAAFGVEVDCSRFPNTTNEEGKDEVVCPDELRLICGTDGVTYNHECMLCFYNKEYGTNISKEQDGECGETVPMDCSRYPNTTSEDGKVTILCTKDFSFVCGTDGVTYDNECMLCAHNIVQGTSVGKKHDGECRKELAAVSVDCSEYPKPACPKDYRPVCGSDNKTYSNKCNFCNAVVESNGTLTLNHFGKC

SEQ ID NO: 19 - protein, 205 aa, Anas platyrhynchos
MAGVFVLLSLVLCCFPDAAFGVEVDCSRFPNTTNEEGKDVLLCTKELSPVCGTDGVTYSNECLLCAYNIEYGTNISKDHDGECKEAVPADCSMYPNMTNEEGKMTLLCNKMFSPVCGTDGVTYDNECMLCAHNVEQGTSVGKKYDGKCKKEVATVDCSGYPKPACTMEYMPLCGSDNKTYGNKCNFCNAVVDSNGTLTLSHFGEC

SEQ ID NO: 20 - protein, 171 aa, Anas platyrhynchos
QVDCSRFPNTTNEEGKEVLLCTKELSPVCGTDGVTYSNECLLCAYNIEYGTNISKDHDGECKEAVPADCSMYPNMTNEEGKMTLLCNKMFSPVCGTDGVTYDNECMLCAHNVEQGTSVGKKYDGKCKKEVATVSVDCSGYPKPACTMEYMPLCGSDNKTYGNKCNFCNAVV

SEQ ID NO: 21 - protein, 207 aa, Tyto alba
MTMPGAFVVLSFVLCCFPDATFGVEVDCSTYPNTTNEEGKEVLVCSKILSPICGTDGVTYSNECLLCANNIEYGTNISKYHDGECKEFVPVNCSRYPNTTNEEGKVMLICNKDLSPVCGTDGVTYDNECLLCAHNLEPGTSVGKKYDGECKKEIATVDCSDYPKPVCSLESMPLCGSDNKTYSNKCNFCNAVVDSNETLTLSHFGKC

SEQ ID NO: 22 - protein, 207 aa, Balearica regulorum
  source 1..207: note = Balearica regulorum gibbericeps
MTMAGVFVLLSFALCCFPDAAFGVEVDCSTYPNTTNEEGKEVLVCTKILSPICGTDGVTYSNECLLCAYNIEYGTNVSKDHDGECKEVVPVDCSRYPNSTNEEGKVVMLCSKDLNPVCGTDGVTYDNECVLCAHNVESGTSVGKKYDGECKKETATVDCSDYPKPACTLEYMPFCGSDSKTYSNKCNFCNAVVDSNGTLTLSHFGKC

SEQ ID NO: 23 - protein, 207 aa, Cathartes aura
MTTAGVFVLLSFALCSFPDAAFGVEVDCSTYPNTTNEEGKEVLVCTKILSPICGTDGVTYSNECLLCAYNIEYGTNVSKDHDGECKEFVPVDCSRYPNTTNEDGKVVLLCNKDLSPICGTDGVTYDNECLLCARNLEPGTSVGKKYDGECKKEIATVDCSDYPKPVCSLEYMPLCGSDSKTYSNKCNFCNAVVDSNGTLTLSHFGKC

SEQ ID NO: 24 - protein, 207 aa, Cuculus canorus
MTTAGVFVLLSFTLCSFPDAAFGVEVDCSPYPNTTNEEGKEVLVCNKILSPICGTDGVTYSNECLLCAYNLEYGTNISKDYDGECKEVAPVDCSRHPNTTNEEGKVELLCNKDLNPICGTNGVTYDNECLLCARNLESGTSIGKKYDGECKKEIATVDCSDYPKPVCTLEEMPLCGSDNKTYGNKCNFCNAVVDSNGTLTLSHFGKC

SEQ ID NO: 25 - protein, 207 aa, Antrostomus carolinensis
MTTAVVFVLLSFALCCFPDAAFGVEVDCSTYPNSTNEEGKDVLVCPKILGPICGTDGVTYSNECLLCAYNIQYGTNVSKDHDGECKEIVPVDCSRYPNTTNEEGKVVFLCNKNFDPVCGTDGDTYDNECMLCARSLEPGTTVGKKHDGECKREIATVDCSDYPKPTCSAEDMPLCGSDSKTYSNKCNFCNAVVDSNGTLTLSRFGKC

SEQ ID NO: 26 - protein, 207 aa, Cariama cristata
MTMTGVFVLLSFAICCFPDAAFGVEVDCSTYPNTTNEEGKEVLVCTKILSPICGTDGVTYSNECLLCAYNIEYGTNVSKDHDGECKEVVPVDCSKYPNTTNEEGKVVLLCSKDLSPVCGTDGVTYDNECLLCARNLEPGSSVGKKYDGECKKEIATIDCSDYPKPVCSLEYMPLCGSDSKTYDNKCNFCNAVVDSNGTLTLSHFGKC

SEQ ID NO: 27 - protein, 207 aa, Pygoscelis adeliae
MTTAGVFVLLSFVLCCFPDAVFGVEVDCSTYPNTTNEEGKEVLVCTKILSPICGTDGVTYSNECLLCAYNIEYGTNVSKDHDGECKEVVPVNCSRYPNTTNEEGKVVLRCSKDLSPVCGTDGVTYDNECLMCARNLEPGAVVGKNYDGECKKEIATVDCSDYPKPVCSLEYMPLCGSDSKTYSNKCNFCNAVVDSNGTLTLSHFGKC

SEQ ID NO: 28 - protein, 207 aa, Nipponia nippon
MTTAGVFVLLSIALCCFPDAAFGVEVDCSAYSNTTSEEGKEVLSCTKILSPICGTDGVTYSNECLLCAYNIEYGTNISKDHDGECKEVVSVDCSRYPNTTNEEGKAVLLCNKDLSPVCGTDGVTYDNECLLCAHNLEPGTSVGKKYDGACKKEIATVDCSDYPKPVCTLEYLPLCGSDSKTYSNKCDFCNAVVDSNGTLTLSHFGKC

SEQ ID NO: 29 - protein, 206 aa, Phaethon lepturus
MTTAGVFVLLSFALCCFPDAAFGVEVDCSTYPNTTNEEGKEVLVCTKILSPICGTDGTTYSNECLLCAYNIEYGTNVSKDHDGECKVVPVDCSKYPNTTNEDGKVVLLCNKALSPICGTDRVTYDNECLMCAHNLEPGTSVGKKHDGECQKEVATVDCSDYPKPVCSLEYMPLCGSDGKTYSNKCNFCNAVVNSNGTLTLSHFEKC

SEQ ID NO: 30 - protein, 213 aa, Melopsittacus undulatus
MTTAGVFVLLSFVLCCFFPDAAFGVEVDCSTYPNTTNEEGKEVLVCAKILSPVCGTDGVTYSNECLLCAHNIENGTNVGKDHDGKCKEAVPVDCSRYPNTTDEEGKVVLLCNKDVSPVCGTDGVTYDNECLLCAHNLEAGTSVDKKNDSECKTEDTTLAAVSVDCSDYPKPVCTLEYLPLCGSDNKTYSNKCRFCNAVVDSNGTLTLSRFGKC

SEQ ID NO: 31 - protein, 207 aa, Podiceps cristatus
MTTAGVFVLLSFALCCSPDAAFGVEVDCSTYPNTTNEEGKEVLACTKILSPICGTDGVTYSNECLLCAYNMEYGTNVSKDHDGKCKEVVPVDCSRYPNTTNEEGKVVLLCNKDLSPVCGTDGVTYDNECLLCARNLEPGASVGKKYDGECKKEIATVDCSDYPKPVCSLEHMPLCGSDSKTYSNKCTFCNAVVDSNGTLTLSHFGKC

SEQ ID NO: 32 - protein, 207 aa, Fulmarus glacialis
MTTAGVFVLLSFALCCFPDAAFGVEVDCSTYPNTTNEEGREVLVCTKILSPICGTDGVTYSNECLLCAYNIEYGTNVSKDHDGECKEVAPVGCSRYPNTTNEEGKVVLLCNKDLSPVCGTDGVTYDNECLLCARHLEPGTSVGKKYDGECKKEIATVDCSDYPKPVCSLEYMPLCGSDSKTYSNKCNFCNAVLDSNGTLTLSHFGKC

SEQ ID NO: 33 - protein, 207 aa, Aptenodytes forsteri
MTTAGVFVLLSFALCCFPDAVFGVEVDCSTYPNTTNEEGKEVLVCTKILSPICGTDGVTYSNECLLCAYNIEYGTNVSKDHDGECKEVVPVDCSRYPNTTNEEGKVVLRCNKDLSPVCGTDGVTYDNECLMCARNLEPGAIVGKKYDGECKKEIATVDCSDYPKPVCSLEYMPLCGSDSKTYSNKCNFCNAVVDSNGTLILSHFGKC

SEQ ID NO: 34 - protein, 207 aa, Pygoscelis adeliae
MTTAGVFVLLSFVLCCFPDAVFGVEVDCSTYPNTTNEEGKEVLVCTKILSPICGTDGVTYSNECLLCAYNIEYGTNVSKDHDGECKEVVPVDCSRYPNTTNEEGKVVLRCSKDLSPVCGTDGVTYDNECLMCARNLEPGAVVGKNYDGECKKEIATVDCSDYPKPVCSLEYMPLCGSDSKTYSNKCNFCNAVVDSNGTLTLSHFGKC

SEQ ID NO: 35 - protein, 282 aa, Aptenodytes forsteri
MSSQNQLPSRCRPLPGSQDLNKYYQPHCTGDRFCWLFYVTVEQFRHCICIYLQLALERPSHEQSGQPADSRNTSTMTTAGVFVLLSFALCCFPDAVFGVEVDCSTYPNTTNEEGKEVLVCTKILSPICGTDGVTYSNECLLCAYNIEYGTNVSKDHDGECKEVVPVDCSRYPNTTNEEGKVVLRCNKDLSPVCGTDGVTYDNECLMCARNLEPGAIVGKKYDGECKKEIATVDCSDYPKPVCSLEYMPLCGSDSKTYSNKCNFCNAVVDSNGTLILSHFGKC

SEQ ID NO: 36 - protein, 193 aa, Antrostomus carolinensis
MTTAVVFVLLSFALCCFPDAAFGVEVDCSTYPNSTNEEGKDVLVCPKILGPICGTDGVTYSNECLLCAYNIQYGTNVSKDHDGECKEIVPVDCSRYPNTTNEEGKVVFLCNKNFDPVCGTDGDTYDNECMLCARSLEPGTTVGKKHDGECKREIATVDCSDYPKPTCSAEDMPLCGSDSKTYSNKCNFCNAVV

SEQ ID NO: 37 - protein, 190 aa, Gallus gallus
EAEAAEVDCSRFPNATDKEGKDVLVCNKDLRPICGTDGVTYTNDCLLCAYSIEFGTNISKEHDGECKETVPMNCSSYANTTSEDGKVMVLCNRAFNPVCGTDGVTYDNECLLCAHKVEQGASVDKRHDGGCRKELAAVSVDCSEYPKPDCTAEDRPLCGSDNKTYGNKCNFCNAVVESNGTLTLSHFGKC

SEQ ID NO: 38 - protein, 199 aa, Gallus gallus
EEGVSLEKREAEAAEVDCSRFPNATDKEGKDVLVCNKDLRPICGTDGVTYTNDCLLCAYSIEFGTNISKEHDGECKETVPMNCSSYANTTSEDGKVMVLCNRAFNPVCGTDGVTYDNECLLCAHKVEQGASVDKRHDGGCRKELAAVSVDCSEYPKPDCTAEDRPLCGSDNKTYGNKCNFCNAVVESNGTLTLSHFGKC

SEQ ID NO: 39 - protein, 275 aa, Gallus gallus
MRFPSIFTAVLFAASSALAAPVNTTTEDETAQIPAEAVIGYSDLEGDFDVAVLPFSNSTNNGLLFINTTIASIAAKEEGVSLEKREAEAAEVDCSRFPNATDKEGKDVLVCNKDLRPICGTDGVTYTNDCLLCAYSIEFGTNISKEHDGECKETVPMNCSSYANTTSEDGKVMVLCNRAFNPVCGTDGVTYDNECLLCAHKVEQGASVDKRHDGGCRKELAAVSVDCSEYPKPDCTAEDRPLCGSDNKTYGNKCNFCNAVVESNGTLTLSHFGKC

SEQ ID NO: 40 - protein, 273 aa, Cathartes aura
MRFPSIFTAVLFAASSALAAPVNTTTEDETAQIPAEAVIGYSDLEGDFDVAVLPFSNSTNNGLLFINTTIASIAAKEEGVSLEKREAEAVEVDCSTYPNTTNEEGKEVLVCTKILSPICGTDGVTYSNECLLCAYNIEYGTNVSKDHDGECKEFVPVDCSRYPNTTNEDGKVVLLCNKDLSPICGTDGVTYDNECLLCARNLEPGTSVGKKYDGECKKEIATVDCSDYPKPVCSLEYMPLCGSDSKTYSNKCNFCNAVVDSNGTLTLSHFGKC

SEQ ID NO: 41 - protein, 188 aa, Cathartes aura
EAEAVEVDCSTYPNTTNEEGKEVLVCTKILSPICGTDGVTYSNECLLCAYNIEYGTNVSKDHDGECKEFVPVDCSRYPNTTNEDGKVVLLCNKDLSPICGTDGVTYDNECLLCARNLEPGTSVGKKYDGECKKEIATVDCSDYPKPVCSLEYMPLCGSDSKTYSNKCNFCNAVVDSNGTLTLSHFGKC

SEQ ID NO: 42 - protein, 206 aa, Calypte anna
MTMAGVFVLLSFILCCFPDTAFGVEVDCSIYPNTTSEEGKEVLVCTETLSPICGSDGVTYNNECQLCAYNVEYGTNVSKDHDGECKEIVPVDCSRYPNTTEEGRVVMLCNKALSPVCGTDGVTYDNECLLCARNLESGTSVGKKFDGECKKEIATVDCTDYPKPVCSLDYMPLCGSDSKTYSNKCNFCNAVMDSNGTLTLNHFGKC

SEQ ID NO: 43 - protein, 272 aa, Calypte anna
MRFPSIFTAVLFAASSALAAPVNTTTEDETAQIPAEAVIGYSDLEGDFDVAVLPFSNSTNNGLLFINTTIASIAAKEEGVSLDKREAEAVEVDCSIYPNTTSEEGKEVLVCTETLSPICGSDGVTYNNECQLCAYNVEYGTNVSKDHDGECKEIVPVDCSRYPNTTEEGRVVMLCNKALSPVCGTDGVTYDNECLLCARNLESGTSVGKKFDGECKKEIATVDCTDYPKPVCSLDYMPLCGSDSKTYSNKCNFCNAVMDSNGTLTLNHFGKC

SEQ ID NO: 44 - protein, 187 aa, Calypte anna
EAEAVEVDCSIYPNTTSEEGKEVLVCTETLSPICGSDGVTYNNECQLCAYNVEYGTNVSKDHDGECKEIVPVDCSRYPNTTEEGRVVMLCNKALSPVCGTDGVTYDNECLLCARNLESGTSVGKKFDGECKKEIATVDCTDYPKPVCSLDYMPLCGSDSKTYSNKCNFCNAVMDSNGTLTLNHFGKC

SEQ ID NO: 45 - protein, 218 aa, Gallus gallus
MRFPSIFTAVLFAASSALAAPVNTTTEDETAQIPAEAVIGYSDLEGDFDVAVLPFSNSTNNGLLFINTTIASIAAKEEGVSLDKREAEAKVFGRCELAAAMKRHGLDNYRGYSLGNWVCAAKFESNFNTQATNRNTDGSTDYGILQINSRWWCNDGRTPGSRNLCNIPCSALLSSDITASVNCAKKIVSDGNGMNAWVAWRNRCKGTDVQAWIRGCRL

SEQ ID NO: 46 - protein, 133 aa, Gallus gallus
EAEAKVFGRCELAAAMKRHGLDNYRGYSLGNWVCAAKFESNFNTQATNRNTDGSTDYGILQINSRWWCNDGRTPGSRNLCNIPCSALLSSDITASVNCAKKIVSDGNGMNAWVAWRNRCKGTDVQAWIRGCRL

SEQ ID NO: 47 - protein, 129 aa, Gallus gallus [sequence omitted]

SEQ ID NO: 48 - protein, 129 aa, Gallus gallus
KVFGRCELAAAMKRHGLDNYRGYSLGNWVCVAKFESNFNTQATNRNTDGSTDYGILQINSRWWCNDGRTPGSRNLCNIPCSALLSSDITASVNCAKKIVSDGNGMSAWVAWRNRCKGTDVQAWIRGCRL

SEQ ID NO: 49 - protein, 130 aa, Homo sapiens
KVFERCELARTLKRLGMDGYRGISLANWMCLAKWESGYNTRATNYNAGDRSTDYGIFQINSRYWCNDGKTPGAVNACHLSCSALLQDNIADAVACAKRVVRDPQGIRAWVAWRNRCQNRDVRQYVQGCGV

SEQ ID NO: 50 - protein, 129 aa, Bos taurus
KVFERCELARTLKKLGLDGYKGVSLANWLCLTKWESSYNTKATNYNPSSESTDYGIFQINSKWWCNDGKTPNAVDGCHVSCRELMENDIAKAVACAKHIVSEQGITAWVAWKSHCRDHDVSSYVEGCTL

SEQ ID NO: 51 - protein, 147 aa, Gallus gallus
MRSLLILVLCFLPLAALGKVFGRCELAAAMKRHGLDNYRGYSLGNWVCAAKFESNFNTQATNRNTDGSTDYGILQINSRWWCNDGRTPGSRNLCNIPCSALLSSDITASVNCAKKIVSDGNGMNAWVAWRNRCKGTDVQAWIRGCRL

SEQ ID NO: 52 - protein, 321 aa, synthetic construct
  REGION 1..321: note = Synthetic Peptide
MAKADGSLLYYNPHNPPRRYYFYMAIFAVSVICVLYGPSQQLSSPKIDASAPAPVKQGPTSVAYVEVNNNSMLNVGKYTLADGGGNAFDVAVIFAANINYDTGTKTAYLHFNENVQRVLDNAVTQIRPLQQQGIKVLLSVLGNHQGAGFANFPSQQAASAFAKQLSDAVAKYGLDGVDFDDEYAEYGNNGTAQPNDSSFVHLVTALRANMPDKIISLYNIGPAASRLSYGGVDVSDKFDYAWNPYYGTWQVPGIALPKAQLSPAAVEIGRTSRSTVADLARRTVDEGYGVYLTYNLDGGDRTADVSAFTRELYGSEAVRTP

SEQ ID NO: 53 - protein, 4 aa, synthetic construct
  REGION 1..4: note = Synthetic Peptide
EAEA